European Patent Application EP 4 219 737 A1, published August 2, 2023. Title: COMBINATION, METHOD AND KIT FOR DETECTING NUCLEIC ACID. Applicant: MACCURA BIOTECHNOLOGY CO., LTD. The sequence listing filed with the application follows.

SEQUENCE LISTING (17 sequences)

SEQ ID NO: 1 - DNA, 40 bp, Artificial sequence
  Artificial sequence
ccgactgctgacaaagtataaaaaagatcaaagtgctggc

SEQ ID NO: 2 - DNA, 17 bp, Artificial sequence
  Artificial sequence
gccgaacgcaccggagg

SEQ ID NO: 3 - DNA, 37 bp, Artificial sequence
  Artificial sequence
ccgcctgtacaggcggtaccgactgctgacaaagtat

SEQ ID NO: 4 - DNA, 63 bp, Artificial sequence
  Artificial sequence
cgacggctgacacgataactctgactcaccacaacgagaattcaaaaagatcaaagtgctggc

SEQ ID NO: 5 - DNA, 17 bp, Artificial sequence
  Artificial sequence
cgacggctgacacgata

SEQ ID NO: 6 - DNA, 18 bp, Artificial sequence
  Artificial sequence
ctctgactcaccacaacg

SEQ ID NO: 7 - DNA, 42 bp, Artificial sequence
  Artificial sequence
ccgactgctgacaaagtataattcaaaaagatcaaagtgctg

SEQ ID NO: 8 - DNA, 39 bp, Artificial sequence
  Artificial sequence
ccgactgctgacaaagtataggatcttgaaggaaactga

SEQ ID NO: 9 - DNA, 41 bp, Artificial sequence
  Artificial sequence
ccgactgctgacaaagtatagctcccaaccaaactctcttg

SEQ ID NO: 10 - DNA, 40 bp, Artificial sequence
  Artificial sequence
ccgactgctgacaaagtatatcttacacccagtggagaag

SEQ ID NO: 11 - DNA, 41 bp, Artificial sequence
  Artificial sequence
ccgactgctgacaaagtatacagcttgtggagcttcttaca

SEQ ID NO: 12 - DNA, 34 bp, Artificial sequence
  Artificial sequence
ccgctgcgcagcggtccaccgtgcarctcataat

SEQ ID NO: 13 - DNA, 18 bp, Artificial sequence
  Artificial sequence
caccgtgcarctcatcac

SEQ ID NO: 14 - DNA, 22 bp, Artificial sequence
  Artificial sequence
cagccgaagggcatgagctgca

SEQ ID NO: 15 - DNA, 18 bp, Artificial sequence
  Artificial sequence
cccggacatagtccagga

SEQ ID NO: 16 - DNA, 18 bp, Artificial sequence
  Artificial sequence
tgagcaggtactgggagc

SEQ ID NO: 17 - DNA, 18 bp, Artificial sequence
  Artificial sequence
ctgattacctttgcgatc